European Patent Application EP 4 578 957 A2, published July 2, 2025. Title: Methods for quantifying drug concentration in a prodrug composition. Applicant: Genzyme Corporation. Application EP. The sequence listing filed with the application follows.

SEQUENCE LISTING (2 sequences)

SEQ ID NO: 1 - protein, 19 aa, synthetic construct
  REGION 1..19: note = source = /note="Description of Artificial Sequence: Synthetic peptide"
DFIEWLKAGGPSSGAPPPS

SEQ ID NO: 2 - protein, 13 aa, synthetic construct
  MOD_RES 7: note = Glu-palm
  REGION 1..13: note = source = /note="Description of Artificial Sequence: Synthetic peptide"
DLSKQKXESKAAQ